European Patent Application EP 4 748 934 A1, published May 27, 2026. Title: DNA aptamer for inhibiting FGFR1. Applicant: Masarykova univerzita. Application EP. The sequence listing filed with the application follows.

SEQUENCE LISTING (6 sequences)

SEQ ID NO: 1 - DNA, 40 bp, Synthetic construct
  source 1..40: mol_type = other DNA
  variation 14: note = N = t or a
gggatacagggctntgtctatggtgtggatggcggatacc

SEQ ID NO: 2 - DNA, 40 bp, synthetic construct
  source 1..40: mol_type = other DNA
gggatacagggctttgtctatggtgtggatggcggatacc

SEQ ID NO: 3 - DNA, 40 bp, synthetic construct
  source 1..40: mol_type = other DNA
gggatacagggctatgtctatggtgtggatggcggatacc

SEQ ID NO: 4 - DNA, 40 bp, synthetic construct; identical to SEQ ID NO: 2
  source 1..40: mol_type = other DNA
  modified_base 9: mod_base = OTHER; note = 2-deoxy-2-fluoroarabinoside guanosine

SEQ ID NO: 5 - DNA, 40 bp, synthetic construct; identical to SEQ ID NO: 3
  source 1..40: mol_type = other DNA
  modified_base 32: mod_base = OTHER; note = 2-deoxy-2-fluoroarabinoside guanosine

SEQ ID NO: 6 - DNA, 76 bp, synthetic construct
  source 1..76: mol_type = other DNA
ataccagcttattcaattgggatacagggctttgtctatggtgtggatggcggataccagatagtaagtgcaatct